European Patent Application EP 4 512 902 A1, published February 26, 2025. Title: construct for introducing a foreign substance and use thereof. Applicant: TOAGOSEI CO., LTD. The sequence listing filed with the application follows.

SEQUENCE LISTING (6 sequences)

SEQ ID NO: 1 - protein, 17 aa, synthetic construct
RSRKYTSWYVALKRWPC

SEQ ID NO: 2 - protein, 14 aa, synthetic construct
RSRKYTSWYVALKR

SEQ ID NO: 3 - protein, 14 aa, synthetic construct
KSKKYTSWYVALKR

SEQ ID NO: 4 - protein, 14 aa, synthetic construct
KSRKYTSWYVALKR

SEQ ID NO: 5 - protein, 14 aa, synthetic construct
RSKKYTSWYVALKR

SEQ ID NO: 6 - protein, 14 aa, synthetic construct
RSRKYTSWYVALKK